European Patent Application EP 4 286 409 A1, published December 6, 2023. Title: Antigen-Binding Protein Targeting Staphylococcus aureus α-Hemolysis and application thereof. Applicant: STARMAB BIOLOGICS (SUZHOU) CO., LTD, STARSHINING BIOLOGICS (SHANGHAI) CO., LTD. The sequence listing filed with the application follows.

SEQUENCE LISTING (70 sequences)

SEQ ID NO: 1 - protein, 9 aa, Artificial Sequence
  A3 CDR3
AGENMRLVT

SEQ ID NO: 2 - protein, 6 aa, Artificial Sequence
  A3 CDR2
NIPGDD

SEQ ID NO: 3 - protein, 7 aa, Artificial Sequence
  A3 CDR1
GFTFSRH

SEQ ID NO: 4 - protein, 25 aa, Artificial Sequence
  A3 FR1
QVQLVESGGGLVQAGGSLTLSCVAS

SEQ ID NO: 5 - protein, 19 aa, Artificial Sequence
  A3 FR2
GMTWVRQAPGKELDYVGEI

SEQ ID NO: 6 - protein, 41 aa, Artificial Sequence
  A3 FR3
VDYDISVKGRFTISRDNAKNTVYLHMTNLKVEDTATYWCAQ

SEQ ID NO: 7 - protein, 11 aa, Artificial Sequence
  A3 FR4
RRQGTQVTVST

SEQ ID NO: 8 - protein, 25 aa, Artificial Sequence
  huA3 FR1， huG1 FR1
QVQLVESGGGLVQPGGSLRLSCAAS

SEQ ID NO: 9 - protein, 19 aa, Artificial Sequence
  huA3 FR2
GMTWVRQAPGKGLEYVGEI

SEQ ID NO: 10 - protein, 41 aa, Artificial Sequence
  huA3 FR3
VDYDISVKGRFTISRDNAKNTLYLQMNSLRAEDTAVYYCAR

SEQ ID NO: 11 - protein, 11 aa, Artificial Sequence
  huA3 FR4
RGQGTLVTVSS

SEQ ID NO: 12 - protein, 118 aa, Artificial Sequence
  A3
QVQLVESGGGLVQAGGSLTLSCVASGFTFSRHGMTWVRQAPGKELDYVGEINIPGDDVDYDISVKGRFTISRDNAKNTVYLHMTNLKVEDTATYWCAQAGENMRLVTRRQGTQVTVST

SEQ ID NO: 13 - protein, 118 aa, Artificial Sequence
  huA3
QVQLVESGGGLVQPGGSLRLSCAASGFTFSRHGMTWVRQAPGKGLEYVGEINIPGDDVDYDISVKGRFTISRDNAKNTLYLQMNSLRAEDTAVYYCARAGENMRLVTRGQGTLVTVSS

SEQ ID NO: 14 - protein, 9 aa, Artificial Sequence
  G1 CDR3
QGANLRQGV

SEQ ID NO: 15 - protein, 6 aa, Artificial Sequence
  G1 CDR2
NIPGTD

SEQ ID NO: 16 - protein, 7 aa, Artificial Sequence
  G1 CDR1
GFTISST

SEQ ID NO: 17 - protein, 25 aa, Artificial Sequence
  G1 FR1
QVQLVESGGDLVQPGGSLTLACEAS

SEQ ID NO: 18 - protein, 19 aa, Artificial Sequence
  G1 FR2
GMTWVRQAPGKELDWVGDI

SEQ ID NO: 19 - protein, 41 aa, Artificial Sequence
  G1 FR3
TDYDISVKGRFTISKDHAKNTVYLQMTSLRPEDTAIYYCAK

SEQ ID NO: 20 - protein, 11 aa, Artificial Sequence
  G1 FR4
QSPGTLVTVSS

SEQ ID NO: 21 - protein, 19 aa, Artificial Sequence
  huG1 FR2
GMTWVRQAPGKGLEWVGDI

SEQ ID NO: 22 - protein, 41 aa, Artificial Sequence
  huG1 FR3
TDYDISVKGRFTISKDHAKNTVYLQMNSLRAEDTAVYYCAK

SEQ ID NO: 23 - protein, 11 aa, Artificial Sequence
  huG1 FR4
QGQGTLVTVSS

SEQ ID NO: 24 - protein, 118 aa, Artificial Sequence
  G1
QVQLVESGGDLVQPGGSLTLACEASGFTISSTGMTWVRQAPGKELDWVGDINIPGTDTDYDISVKGRFTISKDHAKNTVYLQMTSLRPEDTAIYYCAKQGANLRQGVQSPGTLVTVSS

SEQ ID NO: 25 - protein, 118 aa, Artificial Sequence
  huG1
QVQLVESGGGLVQPGGSLRLSCAASGFTISSTGMTWVRQAPGKGLEWVGDINIPGTDTDYDISVKGRFTISKDHAKNTVYLQMNSLRAEDTAVYYCAKQGANLRQGVQGQGTLVTVSS

SEQ ID NO: 26 - protein, 17 aa, Artificial Sequence
  F6 CDR3
YRNFGNFCVMGRYEYDE

SEQ ID NO: 27 - protein, 6 aa, Artificial Sequence
  F6 CDR2
SRSGAS

SEQ ID NO: 28 - protein, 7 aa, Artificial Sequence
  F6 CDR1
GSTLDSY

SEQ ID NO: 29 - protein, 25 aa, Artificial Sequence
  F6 FR1
QVQLVESGGGLAQPGGSLRLSCEAS

SEQ ID NO: 30 - protein, 19 aa, Artificial Sequence
  F6 FR2
TVAWFRQAPGKEREGVSCA

SEQ ID NO: 31 - protein, 41 aa, Artificial Sequence
  F6 FR3
TNYANSVKGRFTISRDNAKNTVYLQMNSLKPEDTGVYYCAA

SEQ ID NO: 32 - protein, 11 aa, Artificial Sequence
  F6 FR4
WGQGTQVTVSS

SEQ ID NO: 33 - protein, 25 aa, Artificial Sequence [sequence omitted]

SEQ ID NO: 34 - protein, 19 aa, Artificial Sequence
  huF6 FR2
TVAWVRQAPGKGLEWVSCA

SEQ ID NO: 35 - protein, 41 aa, Artificial Sequence
  huF6 FR3
TNYANSVKGRFTISRDNSKNTVYLQMNSLRAEDTAVYYCAA

SEQ ID NO: 36 - protein, 11 aa, Artificial Sequence
  huF6 FR4
WGQGTLVTVSS

SEQ ID NO: 37 - protein, 126 aa, Artificial Sequence
  F6
QVQLVESGGGLAQPGGSLRLSCEASGSTLDSYTVAWFRQAPGKEREGVSCASRSGASTNYANSVKGRFTISRDNAKNTVYLQMNSLKPEDTGVYYCAAYRNFGNFCVMGRYEYDEWGQGTQVTVSS

SEQ ID NO: 38 - protein, 126 aa, Artificial Sequence
  huF6
EVQLVESGGGLVQPGGSLRLSCAASGSTLDSYTVAWVRQAPGKGLEWVSCASRSGASTNYANSVKGRFTISRDNSKNTVYLQMNSLRAEDTAVYYCAAYRNFGNFCVMGRYEYDEWGQGTLVTVSS

SEQ ID NO: 39 - protein, 232 aa, Artificial Sequence
  IgG1 Fc
EPKSSDKTHTCPPCPAPELLGGPSVFLFPPKPKDTLYITREPEVTCVVVDVSHEDPEVKFNWYVDGVEVHNAKTKPREEQYNSTYRVVSVLTVLHQDWLNGKEYKCKVSNKALPAPIEKTISKAKGQPREPQVYTLPPSREEMTKNQVSLTCLVKGFYPSDIAVEWESNGQPENNYKTTPPVLDSDGSFFLYSKLTVDKSRWQQGNVFSCSVMHEALHNHYTQKSLSLSPGK

SEQ ID NO: 40 - protein, 10 aa, Artificial Sequence
  A3 CDR2 AbM
EINIPGDDVD

SEQ ID NO: 41 - protein, 10 aa, Artificial Sequence
  A3 CDR1 AbM  combination
GFTFSRHGMT

SEQ ID NO: 42 - protein, 17 aa, Artificial Sequence
  A3 CDR2 Kabat  combination
EINIPGDDVDYDISVKG

SEQ ID NO: 43 - protein, 5 aa, Artificial Sequence
  A3 CDR1 Kabat
RHGMT

SEQ ID NO: 44 - protein, 10 aa, Artificial Sequence
  G1 CDR2 AbM
DINIPGTDTD

SEQ ID NO: 45 - protein, 10 aa, Artificial Sequence
  G1 CDR1 AbM  combination
GFTISSTGMT

SEQ ID NO: 46 - protein, 17 aa, Artificial Sequence
  G1 CDR2 Kabat  combination
DINIPGTDTDYDISVKG

SEQ ID NO: 47 - protein, 5 aa, Artificial Sequence
  G1 CDR1 Kabat
STGMT

SEQ ID NO: 48 - protein, 10 aa, Artificial Sequence
  F6 CDR2 AbM
CASRSGASTN

SEQ ID NO: 49 - protein, 10 aa, Artificial Sequence
  F6 CDR1 AbM  combination
GSTLDSYTVA

SEQ ID NO: 50 - protein, 17 aa, Artificial Sequence
  F6 CDR2 Kabat  combination
CASRSGASTNYANSVKG

SEQ ID NO: 51 - protein, 5 aa, Artificial Sequence
  F6 CDR1 Kabat
SYTVA

SEQ ID NO: 52 - protein, 6 aa, Artificial Sequence
  A3 CDR2; G1 CDR2
  misc_feature (5)..(5): Xaa = Asp or Thr
NIPGXD

SEQ ID NO: 53 - protein, 7 aa, Artificial Sequence
  A3 CDR1; G1 CDR1
  misc_feature (4)..(4): Xaa = Phe or Ile
  misc_feature (6)..(6): Xaa = Arg or Ser
  misc_feature (7)..(7): Xaa = His or Thr
GFTXSXX

SEQ ID NO: 54 - protein, 25 aa, Artificial Sequence
  A3 FR1; huA3 FR1; huG1 FR1; G1 FR1; F6 FR1; huF6 FR1
  misc_feature (1)..(1): Xaa = Glu or Gln
  misc_feature (10)..(10): Xaa = Asp or Gly
  misc_feature (12)..(12): Xaa = Ala or Val
  misc_feature (14)..(14): Xaa = Ala or Pro
  misc_feature (19)..(19): Xaa = Arg or Thr
  misc_feature (21)..(21): Xaa = Ala or Ser
  misc_feature (23)..(23): Xaa = Ala、Glu or Val
XVQLVESGGXLXQXGGSLXLXCXAS

SEQ ID NO: 55 - protein, 19 aa, Artificial Sequence
  A3 FR2; huA3 FR2; G1 FR2; huG1 FR2
  misc_feature (12)..(12): Xaa = Glu or Gly
  misc_feature (14)..(14): Xaa = Asp or Glu
  misc_feature (15)..(15): Xaa = Trp or Tyr
  misc_feature (18)..(18): Xaa = Asp or Glu
GMTWVRQAPGKXLXXVGXI

SEQ ID NO: 56 - protein, 19 aa, Artificial Sequence
  F6 FR2; huF6 FR2
  misc_feature (5)..(5): Xaa = Phe or Val
  misc_feature (12)..(12): Xaa = Glu or Gly
  misc_feature (13)..(13): Xaa = Leu or Arg
  misc_feature (15)..(15): Xaa = Gly or Trp
TVAWXRQAPGKXXEXVSCA

SEQ ID NO: 57 - protein, 41 aa, Artificial Sequence
  A3 FR3; huA3 FR3; G1 FR3; huG1 FR3
  misc_feature (1)..(1): Xaa = Thr or Val
  misc_feature (15)..(15): Xaa = Lys or Arg
  misc_feature (17)..(17): Xaa = His or Asn
  misc_feature (22)..(22): Xaa = Leu or Val
  misc_feature (25)..(25): Xaa = His or Gln
  misc_feature (27)..(27): Xaa = Asn or Thr
  misc_feature (28)..(28): Xaa = Asn or Ser
  misc_feature (30)..(30): Xaa = Lys or Arg
  misc_feature (31)..(31): Xaa = Ala、Pro or Val
  misc_feature (36)..(36): Xaa = Ile、Thr or Val
  misc_feature (38)..(38): Xaa = Trp or Tyr
  misc_feature (41)..(41): Xaa = Lys、Gln or Arg
XDYDISVKGRFTISXDXAKNTXYLXMXXLXXEDTAXYXCAX

SEQ ID NO: 58 - protein, 41 aa, Artificial Sequence
  huF6 FR3; F6 FR3
  misc_feature (18)..(18): Xaa = Ala or Ser
  misc_feature (30)..(30): Xaa = Lys or Arg
  misc_feature (31)..(31): Xaa = Ala or Pro
  misc_feature (35)..(35): Xaa = Ala or Gly
TNYANSVKGRFTISRDNXKNTVYLQMNSLXXEDTXVYYCAA

SEQ ID NO: 59 - protein, 11 aa, Artificial Sequence
  A3 FR4; huA3 FR4; G1 FR4; huG1 FR4; F6 FR4; huF6 FR4
  misc_feature (1)..(1): Xaa = Gln、Arg or Trp
  misc_feature (2)..(2): Xaa = Gly、Arg or Ser
  misc_feature (3)..(3): Xaa = Pro or Gln
  misc_feature (6)..(6): Xaa = Leu or Gln
  misc_feature (11)..(11): Xaa = Ser or Thr
XXXGTXVTVSX

SEQ ID NO: 60 - protein, 118 aa, Artificial Sequence
  A3; huA3; G1; huG1
  misc_feature (10)..(10): Xaa = Asp or Gly
  misc_feature (14)..(14): Xaa = Ala or Pro
  misc_feature (19)..(19): Xaa = Arg or Thr
  misc_feature (21)..(21): Xaa = Ala or Ser
  misc_feature (23)..(23): Xaa = Ala、Glu or Val
  misc_feature (29)..(29): Xaa = Phe or Ile
  misc_feature (31)..(31): Xaa = Arg or Ser
  misc_feature (32)..(32): Xaa = His or Thr
  misc_feature (44)..(44): Xaa = Glu or Gly
  misc_feature (46)..(46): Xaa = Asp or Glu
  misc_feature (47)..(47): Xaa = Trp or Tyr
  misc_feature (50)..(50): Xaa = Asp or Glu
  misc_feature (56)..(56): Xaa = Asp or Thr
  misc_feature (58)..(58): Xaa = Thr or Val
  misc_feature (72)..(72): Xaa = Lys or Arg
  misc_feature (74)..(74): Xaa = His or Asn
  misc_feature (79)..(79): Xaa = Leu or Val
  misc_feature (82)..(82): Xaa = His or Gln
  misc_feature (84)..(84): Xaa = Asn or Thr
  misc_feature (85)..(85): Xaa = Asn or Ser
  misc_feature (87)..(87): Xaa = Lys or Arg
  misc_feature (88)..(88): Xaa = Ala、Pro or Val
  misc_feature (93)..(93): Xaa = Ile、Thr or Val
  misc_feature (95)..(95): Xaa = Trp or Tyr
  misc_feature (98)..(98): Xaa = Lys、Gln or Arg
  misc_feature (99)..(99): Xaa = Ala or Gln
  misc_feature (101)..(101): Xaa = Ala or Glu
  misc_feature (103)..(103): Xaa = Leu or Met
  misc_feature (105)..(105): Xaa = Leu or Gln
  misc_feature (106)..(106): Xaa = Gly or Val
  misc_feature (107)..(107): Xaa = Thr or Val
  misc_feature (108)..(108): Xaa = Gln or Arg
  misc_feature (109)..(109): Xaa = Gly、Arg or Ser
  misc_feature (110)..(110): Xaa = Pro or Gln
  misc_feature (113)..(113): Xaa = Leu or Gln
  misc_feature (118)..(118): Xaa = Ser or Thr
QVQLVESGGXLVQXGGSLXLXCXASGFTXSXXGMTWVRQAPGKXLXXVGXINIPGXDXDYDISVKGRFTISXDXAKNTXYLXMXXLXXEDTAXYXCAXXGXNXRXXXXXXGTXVTVSX

SEQ ID NO: 61 - protein, 126 aa, Artificial Sequence
  F6; huF6
  misc_feature (1)..(1): Xaa = Glu or Gln
  misc_feature (12)..(12): Xaa = Ala or Val
  misc_feature (23)..(23): Xaa = Ala or Glu
  misc_feature (37)..(37): Xaa = Phe or Val
  misc_feature (44)..(44): Xaa = Glu or Gly
  misc_feature (45)..(45): Xaa = Leu or Arg
  misc_feature (47)..(47): Xaa = Gly or Trp
  misc_feature (75)..(75): Xaa = Ala or Ser
  misc_feature (87)..(87): Xaa = Lys or Arg
  misc_feature (88)..(88): Xaa = Ala or Pro
  misc_feature (92)..(92): Xaa = Ala or Gly
  misc_feature (121)..(121): Xaa = Leu or Gln
XVQLVESGGGLXQPGGSLRLSCXASGSTLDSYTVAWXRQAPGKXXEXVSCASRSGASTNYANSVKGRFTISRDNXKNTVYLQMNSLXXEDTXVYYCAAYRNFGNFCVMGRYEYDEWGQGTXVTVSS

SEQ ID NO: 62 - protein, 350 aa, Artificial Sequence
  A3-Fc
QVQLVESGGGLVQAGGSLTLSCVASGFTFSRHGMTWVRQAPGKELDYVGEINIPGDDVDYDISVKGRFTISRDNAKNTVYLHMTNLKVEDTATYWCAQAGENMRLVTRRQGTQVTVSTEPKSSDKTHTCPPCPAPELLGGPSVFLFPPKPKDTLYITREPEVTCVVVDVSHEDPEVKFNWYVDGVEVHNAKTKPREEQYNSTYRVVSVLTVLHQDWLNGKEYKCKVSNKALPAPIEKTISKAKGQPREPQVYTLPPSREEMTKNQVSLTCLVKGFYPSDIAVEWESNGQPENNYKTTPPVLDSDGSFFLYSKLTVDKSRWQQGNVFSCSVMHEALHNHYTQKSLSLSPGK

SEQ ID NO: 63 - protein, 350 aa, Artificial Sequence
  G1-Fc
QVQLVESGGDLVQPGGSLTLACEASGFTISSTGMTWVRQAPGKELDWVGDINIPGTDTDYDISVKGRFTISKDHAKNTVYLQMTSLRPEDTAIYYCAKQGANLRQGVQSPGTLVTVSSEPKSSDKTHTCPPCPAPELLGGPSVFLFPPKPKDTLYITREPEVTCVVVDVSHEDPEVKFNWYVDGVEVHNAKTKPREEQYNSTYRVVSVLTVLHQDWLNGKEYKCKVSNKALPAPIEKTISKAKGQPREPQVYTLPPSREEMTKNQVSLTCLVKGFYPSDIAVEWESNGQPENNYKTTPPVLDSDGSFFLYSKLTVDKSRWQQGNVFSCSVMHEALHNHYTQKSLSLSPGK

SEQ ID NO: 64 - protein, 358 aa, Artificial Sequence
  F6-Fc
QVQLVESGGGLAQPGGSLRLSCEASGSTLDSYTVAWFRQAPGKEREGVSCASRSGASTNYANSVKGRFTISRDNAKNTVYLQMNSLKPEDTGVYYCAAYRNFGNFCVMGRYEYDEWGQGTQVTVSSEPKSSDKTHTCPPCPAPELLGGPSVFLFPPKPKDTLYITREPEVTCVVVDVSHEDPEVKFNWYVDGVEVHNAKTKPREEQYNSTYRVVSVLTVLHQDWLNGKEYKCKVSNKALPAPIEKTISKAKGQPREPQVYTLPPSREEMTKNQVSLTCLVKGFYPSDIAVEWESNGQPENNYKTTPPVLDSDGSFFLYSKLTVDKSRWQQGNVFSCSVMHEALHNHYTQKSLSLSPGK

SEQ ID NO: 65 - protein, 483 aa, Artificial Sequence
  huA3-huA3-Fc
QVQLVESGGGLVQPGGSLRLSCAASGFTFSRHGMTWVRQAPGKGLEYVGEINIPGDDVDYDISVKGRFTISRDNAKNTLYLQMNSLRAEDTAVYYCARAGENMRLVTRGQGTLVTVSSGGGGSGGGGSGGGGSQVQLVESGGGLVQPGGSLRLSCAASGFTFSRHGMTWVRQAPGKGLEYVGEINIPGDDVDYDISVKGRFTISRDNAKNTLYLQMNSLRAEDTAVYYCARAGENMRLVTRGQGTLVTVSSEPKSSDKTHTCPPCPAPELLGGPSVFLFPPKPKDTLYITREPEVTCVVVDVSHEDPEVKFNWYVDGVEVHNAKTKPREEQYNSTYRVVSVLTVLHQDWLNGKEYKCKVSNKALPAPIEKTISKAKGQPREPQVYTLPPSREEMTKNQVSLTCLVKGFYPSDIAVEWESNGQPENNYKTTPPVLDSDGSFFLYSKLTVDKSRWQQGNVFSCSVMHEALHNHYTQKSLSLSPGK

SEQ ID NO: 66 - protein, 483 aa, Artificial Sequence
  huG1-huG1-Fc
QVQLVESGGGLVQPGGSLRLSCAASGFTISSTGMTWVRQAPGKGLEWVGDINIPGTDTDYDISVKGRFTISKDHAKNTVYLQMNSLRAEDTAVYYCAKQGANLRQGVQGQGTLVTVSSGGGGSGGGGSGGGGSQVQLVESGGGLVQPGGSLRLSCAASGFTISSTGMTWVRQAPGKGLEWVGDINIPGTDTDYDISVKGRFTISKDHAKNTVYLQMNSLRAEDTAVYYCAKQGANLRQGVQGQGTLVTVSSEPKSSDKTHTCPPCPAPELLGGPSVFLFPPKPKDTLYITREPEVTCVVVDVSHEDPEVKFNWYVDGVEVHNAKTKPREEQYNSTYRVVSVLTVLHQDWLNGKEYKCKVSNKALPAPIEKTISKAKGQPREPQVYTLPPSREEMTKNQVSLTCLVKGFYPSDIAVEWESNGQPENNYKTTPPVLDSDGSFFLYSKLTVDKSRWQQGNVFSCSVMHEALHNHYTQKSLSLSPGK

SEQ ID NO: 67 - protein, 483 aa, Artificial Sequence
  huA3-huG1-Fc
QVQLVESGGGLVQPGGSLRLSCAASGFTFSRHGMTWVRQAPGKGLEYVGEINIPGDDVDYDISVKGRFTISRDNAKNTLYLQMNSLRAEDTAVYYCARAGENMRLVTRGQGTLVTVSSGGGGSGGGGSGGGGSQVQLVESGGGLVQPGGSLRLSCAASGFTISSTGMTWVRQAPGKGLEWVGDINIPGTDTDYDISVKGRFTISKDHAKNTVYLQMNSLRAEDTAVYYCAKQGANLRQGVQGQGTLVTVSSEPKSSDKTHTCPPCPAPELLGGPSVFLFPPKPKDTLYITREPEVTCVVVDVSHEDPEVKFNWYVDGVEVHNAKTKPREEQYNSTYRVVSVLTVLHQDWLNGKEYKCKVSNKALPAPIEKTISKAKGQPREPQVYTLPPSREEMTKNQVSLTCLVKGFYPSDIAVEWESNGQPENNYKTTPPVLDSDGSFFLYSKLTVDKSRWQQGNVFSCSVMHEALHNHYTQKSLSLSPGK

SEQ ID NO: 68 - protein, 350 aa, Artificial Sequence
  HuA3-Fc
QVQLVESGGGLVQPGGSLRLSCAASGFTFSRHGMTWVRQAPGKGLEYVGEINIPGDDVDYDISVKGRFTISRDNAKNTLYLQMNSLRAEDTAVYYCARAGENMRLVTRGQGTLVTVSSEPKSSDKTHTCPPCPAPELLGGPSVFLFPPKPKDTLYITREPEVTCVVVDVSHEDPEVKFNWYVDGVEVHNAKTKPREEQYNSTYRVVSVLTVLHQDWLNGKEYKCKVSNKALPAPIEKTISKAKGQPREPQVYTLPPSREEMTKNQVSLTCLVKGFYPSDIAVEWESNGQPENNYKTTPPVLDSDGSFFLYSKLTVDKSRWQQGNVFSCSVMHEALHNHYTQKSLSLSPGK

SEQ ID NO: 69 - protein, 350 aa, Artificial Sequence
  HuG1-Fc
QVQLVESGGGLVQPGGSLRLSCAASGFTISSTGMTWVRQAPGKGLEWVGDINIPGTDTDYDISVKGRFTISKDHAKNTVYLQMNSLRAEDTAVYYCAKQGANLRQGVQGQGTLVTVSSEPKSSDKTHTCPPCPAPELLGGPSVFLFPPKPKDTLYITREPEVTCVVVDVSHEDPEVKFNWYVDGVEVHNAKTKPREEQYNSTYRVVSVLTVLHQDWLNGKEYKCKVSNKALPAPIEKTISKAKGQPREPQVYTLPPSREEMTKNQVSLTCLVKGFYPSDIAVEWESNGQPENNYKTTPPVLDSDGSFFLYSKLTVDKSRWQQGNVFSCSVMHEALHNHYTQKSLSLSPGK

SEQ ID NO: 70 - protein, 358 aa, Artificial Sequence
  HuF6-Fc
EVQLVESGGGLVQPGGSLRLSCAASGSTLDSYTVAWVRQAPGKGLEWVSCASRSGASTNYANSVKGRFTISRDNSKNTVYLQMNSLRAEDTAVYYCAAYRNFGNFCVMGRYEYDEWGQGTLVTVSSEPKSSDKTHTCPPCPAPELLGGPSVFLFPPKPKDTLYITREPEVTCVVVDVSHEDPEVKFNWYVDGVEVHNAKTKPREEQYNSTYRVVSVLTVLHQDWLNGKEYKCKVSNKALPAPIEKTISKAKGQPREPQVYTLPPSREEMTKNQVSLTCLVKGFYPSDIAVEWESNGQPENNYKTTPPVLDSDGSFFLYSKLTVDKSRWQQGNVFSCSVMHEALHNHYTQKSLSLSPGK